European Patent Application EP 4 596 698 A1, published August 6, 2025. Title: TARGETING VECTOR, PREPARATION METHOD THEREFOR, AND USE THEREOF. Applicant: Shenzhen Genocury Biotech Co., Ltd. Application WO PCT/CN2023/122954, filed September 28, 2023. The sequence listing filed with the application follows.

SEQUENCE LISTING (23 sequences)

SEQ ID NO: 1 - protein, 21 aa, unidentified
MALPVTALLLPLALLLHAARP

SEQ ID NO: 2 - protein, 117 aa, unidentified
EVQLVESGGGLVKPGGSLKLSCAASGLTFSSYAMSWVRQTPEKRLEWVASISSGGFTYYPDSVKGRFTISRDNARNILYLQMSSLRSEDTAMYYCARDEVRGYLDVWGAGTTVTVSS

SEQ ID NO: 3 - protein, 15 aa, unidentified
GGGGSGGGGSGGGGS

SEQ ID NO: 4 - protein, 112 aa, unidentified
AAYKDIQMTQTTSSLSASLGDRVTISCSASQGISNYLNWYQQKPDGTVKLLIYYTSSLHSGVPSRFSGSGSGTDYSLTISNLEPEDIATYYCQQYSKLPYTFGGGTKLEIKR

SEQ ID NO: 5 - protein, 45 aa, unidentified
TTTPAPRPPTPAPTIASQPLSLRPEACRPAAGGAVHTRGLDFACD

SEQ ID NO: 6 - protein, 24 aa, unidentified
IYIWAPLAGTCGVLLLSLVITLYC

SEQ ID NO: 7 - protein, 495 aa, Vesicular Stomatitis Virus-Indiana
KFTIVFPHNQKGNWKNVPSNYHYCPSSSDLNWHNDLIGTALQVKMPKSHKAIQADGWMCHASKWVTTCDFRWYGPKYITHSIRSFTPSVEQCKESIEQTKQGTWLNPGFPPQSCGYATVTDAEAVIVQVTPHHVLVDEYTGEWVDSQFINGKCSNYICPTVHNSTTWHSDYKVKGLCDSNLISMDITFFSEDGELSSLGKEGTGFRSNYFAYETGGKACKMQYCKHWGVRLPSGVWFEMADKDLFAAARFPECPEGSSISAPSQTSVDVSLIQDVERILDYSLCQETWSKIRAGLPISPVDLSYLAPKNPGTGPAFTIINGTLKYFETRYIRVDIAAPILSRMVGMISGTTTERELWDDWAPYEDVEIGPNGVLRTSSGYKFPLYMIGHGMLDSDLHLSSKAQVFEHPHIQDAASQLPDDESLFFGDTGLSKNPIELVEGWFSSWKSSIASFFFIIGLIIGLFLVLRVGIHLCIKLKHTKKRQIYTDIEMNRLGK

SEQ ID NO: 8 - protein, 495 aa, synthetic construct
KFTIVFPHNQKGNWKNVPSNYHYCPSSSDLNWHNDLIGTALQVKMPKSHKAIQADGWMCHASKWVTTCDFRWYGPKYITHSIRSFTPSVEQCKESIEQTKQGTWLNPGFPPQSCGYATVTDAEAVIVQVTPHHVLVDEYTGEWVDSQFINGKCSNYICPTVHNSTTWHSDYKVKGLCDSNLISMDITFFSEDGELSSLGKEGTGFRSNYFAYETGGKACKMQYCKHWGVRLPSGVWFEMADKDLFAAARFPECPEGSSISAPSQTSVDVSLIQDVERILDYSLCQETWSKIRAGLPISPVDLSYLAPKNPGTGPAFTIINGTLKYFETRYIRVDIAAPILSRMVGMISGTTTEQELWDDWAPYEDVEIGPNGVLRTSSGYKFPLYMIGHGMLDSDLHLSSKAQVFEHPHIQDAASQLPDDESLFFGDTGLSKNPIELVEGWFSSWKSSIASFFFIIGLIIGLFLVLRVGIHLCIKLKHTKKRQIYTDIEMNRLGK

SEQ ID NO: 9 - protein, 218 aa, unidentified
DIQLTQSPSTLSASVGDRVTITCRASESLDNYGIRFLTWFQQKPGKAPKLLMYAASNQGSGVPSRFSGSGSGTEFTLTISSLQPDDFATYYCQQTKEVPWSFGQGTKVEVKRTVAAPSVFIFPPSDEQLKSGTASVVCLLNNFYPREAKVQWKVDNALQSGNSQESVTEQDSKDSTYSLSSTLTLSKADYEKHKVYACEVTHQGLSSPVTKSFNRGEC

SEQ ID NO: 10 - protein, 443 aa, unidentified
EVQLVQSGAEVKKPGSSVKVSCKASGYTITDSNIHWVRQAPGQSLEWIGYIYPYNGGTDYNQKFKNRATLTVDNPTNTAYMELSSLRSEDTAFYYCVNGNPWLAYWGQGTLVTVSSASTKGPSVFPLAPCSRSTSESTAALGCLVKDYFPEPVTVSWNSGALTSGVHTFPAVLQSSGLYSLSSVVTVPSSSLGTKTYTCNVDHKPSNTKVDKRVESKYGPPCPPCPAPEFLGGPSVFLFPPKPKDTLMISRTPEVTCVVVDVSQEDPEVQFNWYVDGVEVHNAKTKPREEQFNSTYRVVSVLTVLHQDWLNGKEYKCKVSNKGLPSSIEKTISKAKGQPREPQVYTLPPSQEEMTKNQVSLTCLVKGFYPSDIAVEWESNGQPENNYKTTPPVLDSDGSFFLYSRLTVDKSRWQEGNVFSCSVMHEALHNHYTQKSLSLSLGK

SEQ ID NO: 11 - protein, 120 aa, unidentified
EVKLQESGPGLVAPSQSLSVTCTVSGVSLPDYGVSWIRQPPRKGLEWLGVIWGSETTYYNSALKSRLTIIKDNSKSQVFLKMNSLQTDDTAIYYCAKHYYYGGSYAMDYWGQGTSVTVSS

SEQ ID NO: 12 - protein, 107 aa, unidentified
DIQMTQTTSSLSASLGDRVTISCRASQDISKYLNWYQQKPDGTVKLLIYHTSRLHSGVPSRFSGSGSGTDYSLTISNLEQEDIATYFCQQGNTLPYTFGGGTKLEIT

SEQ ID NO: 13 - protein, 110 aa, unidentified
DIVLTQPPSASGTPGQRVTISCTGSSSGIGNAYVSWYQQLPGKAPKLLIYKNGQRPSGVSDRFSGSKSGTSASLAISGLRSEDEADYYCAAWDDSLNGWVFGGGTKVTVL

SEQ ID NO: 14 - protein, 123 aa, unidentified
MAEVQLLESGGGLVQPGGSLRLSCAASGFTFSDYYMSWVRQAPGKGLEWVSAITTGGGSPNYADSVKGRFTISRDNSKNTLYLQMNSLRAEDTAVYYCARDRTAGYFDYWGQGALVTVSSGSA

SEQ ID NO: 15 - protein, 214 aa, unidentified
DIQMTQSPSSLSASVGDRVTITCKASQDVSIGVAWYQQKPGKAPKLLIYSASYRYTGVPSRFSGSGSGTDFTLTISSLQPEDFATYYCQQYYIYPYTFGQGTKVEIKRTVAAPSVFIFPPSDEQLKSGTASVVCLLNNFYPREAKVQWKVDNALQSGNSQESVTEQDSKDSTYSLSSTLTLSKADYEKHKVYACEVTHQGLSSPVTKSFNRGEC

SEQ ID NO: 16 - protein, 448 aa, unidentified
EVQLVESGGGLVQPGGSLRLSCAASGFTFTDYTMDWVRQAPGKGLEWVADVNPNSGGSIYNQRFKGRFTLSVDRSKNTLYLQMNSLRAEDTAVYYCARNLGPSFYFDYWGQGTLVTVSSASTKGPSVFPLAPSSKSTSGGTAALGCLVKDYFPEPVTVSWNSGALTSGVHTFPAVLQSSGLYSLSSVVTVPSSSLGTQTYICNVNHKPSNTKVDKKVEPKSCDKTHTCPPCPAPELLGGPSVFLFPPKPKDTLMISRTPEVTCVVVDVSHEDPEVKFNWYVDGVEVHNAKTKPREEQYNSTYRVVSVLTVLHQDWLNGKEYKCKVSNKALPAPIEKTISKAKGQPREPQVYTLPPSREEMTKNQVSLTCLVKGFYPSDIAVEWESNGQPENNYKTTPPVLDSDGSFFLYSKLTVDKSRWQQGNVFSCSVMHEALHNHYTQKSLSLSPG

SEQ ID NO: 17 - protein, 122 aa, unidentified
MQVQLQQSGPELEKPGASVKISCKASGYSFTGYTMNWVKQSHGKSLEWIGLITPYNGASSYNQKFRGKATLTVDKSSSTAYMDLLSLTSEDSAVYFCARGGYDGRGFDYWGQGTTVTVSSGV

SEQ ID NO: 18 - protein, 106 aa, unidentified
DIELTQSPAIMSASPGEKVTMTCSASSSVSYMHWYQQKSGTSPKRWIYDTSKLASGVPGRFSGSGSGNSYSLTISSVEAEDDATYYCQQWSGYPLTFGAGTKLEIK

SEQ ID NO: 19 - protein, 118 aa, unidentified
EVQLVESGGGLVQPGGSLRLSCAASGFNIKDTYIHFVRQAPGKGLEWIGRIDPANDNTLYASKFQGKATISADTSKNTAYLQMNSLRAEDTAVYYCGRGYGYYVFDHWGQGTLVTVSS

SEQ ID NO: 20 - protein, 107 aa, unidentified
DVQITQSPSSLSASVGDRVTITCRTSRSISQYLAWYQQKPGKVPKLLIYSGSTLQSGVPSRFSGSGSGTDFTLTISSLQPEDVATYYCQQHNENPLTFGGGTKVEIK

SEQ ID NO: 21 - protein, 494 aa, synthetic construct
KFTIVFPHNQKGNWKNVPSNYHYCPSSSDLNWHNDLIGTALQVKMPSHKAIQADGWMCHASKWVTTCDFRWYGPKYITHSIRSFTPSVEQCKESIEQTKQGTWLNPGFPPQSCGYATVTDAEAVIVQVTPHHVLVDEYTGEWVDSQFINGKCSNYICPTVHNSTTWHSDYKVKGLCDSNLISMDITFFSEDGELSSLGKEGTGFRSNYFAYETGGKACKMQYCKHWGVRLPSGVWFEMADKDLFAAARFPECPEGSSISAPSQTSVDVSLIQDVERILDYSLCQETWSKIRAGLPISPVDLSYLAPKNPGTGPAFTIINGTLKYFETRYIRVDIAAPILSRMVGMISGTTTERELWDDWAPYEDVEIGPNGVLRTSSGYKFPLYMIGHGMLDSDLHLSSKAQVFEHPHIQDAASQLPDDESLFFGDTGLSKNPIELVEGWFSSWKSSIASFFFIIGLIIGLFLVLRVGIHLCIKLKHTKKRQIYTDIEMNRLGK

SEQ ID NO: 22 - protein, 494 aa, synthetic construct
KFTIVFPHNQKGNWKNVPSNYHYCPSSSDLNWHNDLIGTALQVKMPKSHKAIQADGWMCHASKWVTTCDFRWYGPKYITHSIRSFTPSVEQCKESIEQTKQGTWLNPGFPPQSCGYATVTDAEAVIVQVTPHHVLVDEYTGEWVDSQFINGKCSNYICPTVHNSTTWHSDYKVKGLCDSNLISMDITFFSEDGELSSLGKEGTGFRSNYFAYETGGKACKMQYCKHWGVRLPSGVWFEMADKDLFAAARFPECPEGSSISAPSQTSVDVSLIQDVERILDYSLCQETWSKIRAGLPISPVDLSYLAPKNPGTGPAFTIINGTLKYFETRYIRVDIAAPILSRMVGMISGTTTEELWDDWAPYEDVEIGPNGVLRTSSGYKFPLYMIGHGMLDSDLHLSSKAQVFEHPHIQDAASQLPDDESLFFGDTGLSKNPIELVEGWFSSWKSSIASFFFIIGLIIGLFLVLRVGIHLCIKLKHTKKRQIYTDIEMNRLGK

SEQ ID NO: 23 - protein, 495 aa, synthetic construct
KFTIVFPHNQKGNWKNVPSNYHYCPSSSDLNWHNDLIGTALQVKMPQSHKAIQADGWMCHASKWVTTCDFRWYGPKYITHSIRSFTPSVEQCKESIEQTKQGTWLNPGFPPQSCGYATVTDAEAVIVQVTPHHVLVDEYTGEWVDSQFINGKCSNYICPTVHNSTTWHSDYKVKGLCDSNLISMDITFFSEDGELSSLGKEGTGFRSNYFAYETGGKACKMQYCKHWGVRLPSGVWFEMADKDLFAAARFPECPEGSSISAPSQTSVDVSLIQDVERILDYSLCQETWSKIRAGLPISPVDLSYLAPKNPGTGPAFTIINGTLKYFETRYIRVDIAAPILSRMVGMISGTTTERELWDDWAPYEDVEIGPNGVLRTSSGYKFPLYMIGHGMLDSDLHLSSKAQVFEHPHIQDAASQLPDDESLFFGDTGLSKNPIELVEGWFSSWKSSIASFFFIIGLIIGLFLVLRVGIHLCIKLKHTKKRQIYTDIEMNRLGK